European Patent Specification EP 3 290 514 B1, published February 26, 2025. Title: Application of PI4KIIIA protein and related membrane protein complex in treating Alzheimer's disease. Applicant: JIANGSU NUO-BETA PHARMACEUTICAL TECHNOLOGY CO., LTD. Application EP 16785990.9. The sequence listing filed with the application follows.

SEQUENCE LISTING (6 sequences)

SEQ ID NO: 1 - protein, 65 aa, Drosophila melanogaster
MASKVSILLLLTVHLLAAQTFAQDAEFRHDSGYEVHHQKLVFFAEDVGSNKGAIIGLMVGGVVIA

SEQ ID NO: 2 - protein, 24 aa, Ratus norvegicus
MAQFLRLCIWLLALGSCLLATVQA

SEQ ID NO: 3 - protein, 17 aa, Artificial sequence
KRSNRSKRLQYQKDSYC

SEQ ID NO: 4 - DNA, 21 bp, Artificial sequence
aggtatcattcaggttctgtt

SEQ ID NO: 5 - DNA, 19 bp, Artificial sequence
ggttattgaaattcgaact

SEQ ID NO: 6 - DNA, 19 bp, Artificial sequence
tgctcattagcagtaaaga